European Patent Application EP 4 242 222 A1, published September 13, 2023. Title: CHIMERIC PROTEIN COMPRISING THE RECEPTOR BINDING DOMAIN OF THE CORONAVIRUS SPIKE PROTEIN AND COMPOSITIONS THEREOF. Applicant: CENTRO DE INGENIERIA GENETICA Y BIOTECNOLOGIA. The sequence listing filed with the application follows.

SEQUENCE LISTING (11 sequences)

SEQ ID NO: 1 - protein, 201 aa, Artificial Sequence
  Oligonucleotide for aplification pPICZalfaA vector
NITNLCPFGEVFNATRFASVYAWNRKRISNCVADYSVLYNSASFSTFKCYGVSPTKLNDLCFTNVYADSFVIRGDEVRQIAPGQTGKIADYNYKLPDDFTGCVIAWNSNNLDSKVGGNYNYLYRLFRKSNLKPFERDISTEIYQAGSTPCNGVEGFNCYFPLQSYGFQPTNGVGYQPYRVVVLSFELLHAPATVCGPKKST

SEQ ID NO: 2 - protein, 207 aa, Artificial Sequence
  Amino acidic sequence of the RBDH protein
NITNLCPFGEVFNATRFASVYAWNRKRISNCVADYSVLYNSASFSTFKCYGVSPTKLNDLCFTNVYADSFVIRGDEVRQIAPGQTGKIADYNYKLPDDFTGCVIAWNSNNLDSKVGGNYNYLYRLFRKSNLKPFERDISTEIYQAGSTPCNGVEGFNCYFPLQSYGFQPTNGVGYQPYRVVVLSFELLHAPATVCGPKKSTHHHHHH

SEQ ID NO: 3 - protein, 222 aa, Artificial Sequence
  Amino acidic sequence of  RBDcmycH protein
NITNLCPFGEVFNATRFASVYAWNRKRISNCVADYSVLYNSASFSTFKCYGVSPTKLNDLCFTNVYADSFVIRGDEVRQIAPGQTGKIADYNYKLPDDFTGCVIAWNSNNLDSKVGGNYNYLYRLFRKSNLKPFERDISTEIYQAGSTPCNGVEGFNCYFPLQSYGFQPTNGVGYQPYRVVVLSFELLHAPATVCGPKKSREQKLISEEDLNSAVDHHHHHH

SEQ ID NO: 4 - protein, 237 aa, Artificial Sequence
  Amino acidic sequece of CRBDH6-P protein
NWSFFSNIGGSSGGSNITNLCPFGEVFNATRFASVYAWNRKRISNCVADYSVLYNSASFSTFKCYGVSPTKLNDLCFTNVYADSFVIRGDEVRQIAPGQTGKIADYNYKLPDDFTGCVIAWNSNNLDSKVGGNYNYLYRLFRKSNLKPFERDISTEIYQAGSTPCNGVEGFNCYFPLQSYGFQPTNGVGYQPYRVVVLSFELLHAPATVCGPKKGGSGGSSSSSSSSSSIEHHHHHH

SEQ ID NO: 5 - protein, 227 aa, Artificial Sequence
  Amino acidic sequence of CRBDH6-H protein
WSFFSNIGGSGGRFPNITNLCPFGEVFNATRFASVYAWNRKRISNCVADYSVLYNSASFSTFKCYGVSPTKLNDLCFTNVYADSFVIRGDEVRQIAPGQTGKIADYNYKLPDDFTGCVIAWNSNNLDSKVGGNYNYLYRLFRKSNLKPFERDISTEIYQAGSTPCNGVEGFNCYFPLQSYGFQPTNGVGYQPYRVVVLSFELLHAPATVCGPKKSTNLAAAHHHHHH

SEQ ID NO: 6 - protein, 209 aa, Artificial Sequence
  Amino acidic sequence of CRBD protein
NWSFFSNINITNLCPFGEVFNATRFASVYAWNRKRISNCVADYSVLYNSASFSTFKCYGVSPTKLNDLCFTNVYADSFVIRGDEVRQIAPGQTGKIADYNYKLPDDFTGCVIAWNSNNLDSKVGGNYNYLYRLFRKSNLKPFERDISTEIYQAGSTPCNGVEGFNCYFPLQSYGFQPTNGVGYQPYRVVVLSFELLHAPATVCGPKKST

SEQ ID NO: 7 - DNA, 32 bp, Artificial Sequence
  Oligonucleotide for apmplification pPICZalfaA vector
gcatgctcttcagtttgtagccttagacatga

SEQ ID NO: 8 - DNA, 33 bp, Artificial Sequence
  Oligonucleotide used for amplification pPICZalfaA vector
gcatgctcttcttgcttcagcctctctcttctc

SEQ ID NO: 9 - protein, 19 aa, Artificial Sequence
  Amino acidic signal peptide sequence of the LRP1 human protein
MLTPPLLLLLPLLSALVAA

SEQ ID NO: 10 - protein, 222 aa, Artificial Sequence
  Amino acidic sequence of the RBDH6-P protein
NITNLCPFGEVFNATRFASVYAWNRKRISNCVADYSVLYNSASFSTFKCYGVSPTKLNDLCFTNVYADSFVIRGDEVRQIAPGQTGKIADYNYKLPDDFTGCVIAWNSNNLDSKVGGNYNYLYRLFRKSNLKPFERDISTEIYQAGSTPCNGVEGFNCYFPLQSYGFQPTNGVGYQPYRVVVLSFELLHAPATVCGPKKGGSGGSSSSSSSSSSIEHHHHHH

SEQ ID NO: 11 - protein, 215 aa, Artificial Sequence
  Amino acidic sequence of the RBDH6-H protein
RFPNITNLCPFGEVFNATRFASVYAWNRKRISNCVADYSVLYNSASFSTFKCYGVSPTKLNDLCFTNVYADSFVIRGDEVRQIAPGQTGKIADYNYKLPDDFTGCVIAWNSNNLDSKVGGNYNYLYRLFRKSNLKPFERDISTEIYQAGSTPCNGVEGFNCYFPLQSYGFQPTNGVGYQPYRVVVLSFELLHAPATVCGPKKSTNLAAAHHHHHH